European Patent Application EP 4 123 019 A1, published January 25, 2023. Title: Exosomes derived from umbilical cord blood plasma or their mimics and pharmaceutical use of thereof. Applicant: CATHOLIC UNIVERSITY INDUSTRY ACADEMIC COOPERATION FOUNDATION. The sequence listing filed with the application follows.

SEQUENCE LISTING (18 sequences)

SEQ ID NO: 1 - DNA, 2387 bp, Artificial Sequence
  Homo sapiens matrix metallopeptidase 9 (MMP9)
agacacctctgccctcaccatgagcctctggcagcccctggtcctggtgctcctggtgctgggctgctgctttgctgcccccagacagcgccagtccacccttgtgctcttccctggagacctgagaaccaatctcaccgacaggcagctggcagaggaatacctgtaccgctatggttacactcgggtggcagagatgcgtggagagtcgaaatctctggggcctgcgctgctgcttctccagaagcaactgtccctgcccgagaccggtgagctggatagcgccacgctgaaggccatgcgaaccccacggtgcggggtcccagacctgggcagattccaaacctttgagggcgacctcaagtggcaccaccacaacatcacctattggatccaaaactactcggaagacttgccgcgggcggtgattgacgacgcctttgcccgcgccttcgcactgtggagcgcggtgacgccgctcaccttcactcgcgtgtacagccgggacgcagacatcgtcatccagtttggtgtcgcggagcacggagacgggtatcccttcgacgggaaggacgggctcctggcacacgcctttcctcctggccccggcattcagggagacgcccatttcgacgatgacgagttgtggtccctgggcaagggcgtcgtggttccaactcggtttggaaacgcagatggcgcggcctgccacttccccttcatcttcgagggccgctcctactctgcctgcaccaccgacggtcgctccgacggcttgccctggtgcagtaccacggccaactacgacaccgacgaccggtttggcttctgccccagcgagagactctacacccaggacggcaatgctgatgggaaaccctgccagtttccattcatcttccaaggccaatcctactccgcctgcaccacggacggtcgctccgacggctaccgctggtgcgccaccaccgccaactacgaccgggacaagctcttcggcttctgcccgacccgagctgactcgacggtgatggggggcaactcggcgggggagctgtgcgtcttccccttcactttcctgggtaaggagtactcgacctgtaccagcgagggccgcggagatgggcgcctctggtgcgctaccacctcgaactttgacagcgacaagaagtggggcttctgcccggaccaaggatacagtttgttcctcgtggcggcgcatgagttcggccacgcgctgggcttagatcattcctcagtgccggaggcgctcatgtaccctatgtaccgcttcactgaggggccccccttgcataaggacgacgtgaatggcatccggcacctctatggtcctcgccctgaacctgagccacggcctccaaccaccaccacaccgcagcccacggctcccccgacggtctgccccaccggaccccccactgtccacccctcagagcgccccacagctggccccacaggtcccccctcagctggccccacaggtccccccactgctggcccttctacggccactactgtgcctttgagtccggtggacgatgcctgcaacgtgaacatcttcgacgccatcgcggagattgggaaccagctgtatttgttcaaggatgggaagtactggcgattctctgagggcagggggagccggccgcagggccccttccttatcgccgacaagtggcccgcgctgccccgcaagctggactcggtctttgaggagcggctctccaagaagcttttcttcttctctgggcgccaggtgtgggtgtacacaggcgcgtcggtgctgggcccgaggcgtctggacaagctgggcctgggagccgacgtggcccaggtgaccggggccctccggagtggcagggggaagatgctgctgttcagcgggcggcgcctctggaggttcgacgtgaaggcgcagatggtggatccccggagcgccagcgaggtggaccggatgttccccggggtgcctttggacacgcacgacgtcttccagtaccgagagaaagcctatttctgccaggaccgcttctactggcgcgtgagttcccggagtgagttgaaccaggtggaccaagtgggctacgtgacctatgacatcctgcagtgccctgaggactagggctcccgtcctgctttggcagtgccatgtaaatccccactgggaccaaccctggggaaggagccagtttgccggatacaaactggtattctgttctggaggaaagggaggagtggaggtgggctgggccctctcttctcacctttgttttttgttggagtgtttctaataaacttggattctctaacctttaaaaaaaaaaaaaaaaaaaaaaaaaaaaaaaaaaaaaaaaaaaaaaaaaaaa

SEQ ID NO: 2 - DNA, 515 bp, Artificial Sequence
  Homo sapiens galectin 7 (LGALS7)
acggctgcccaacccggtcccagccatgtccaacgtcccccacaagtcctcactgcccgagggcatccgccctggcacggtgctgagaattcgcggcttggttcctcccaatgccagcaggttccatgtaaacctgctgtgcggggaggagcagggctccgatgccgcgctgcatttcaacccccggctggacacgtcggaggtggtcttcaacagcaaggagcaaggctcctggggccgcgaggagcgcgggccgggcgttcctttccagcgcgggcagcccttcgaggtgctcatcatcgcgtcagacgacggcttcaaggccgtggttggggacgcccagtaccaccacttccgccaccgcctgccgctggcgcgcgtgcgcctggtggaggtgggcggggacgtgcagctggactccgtgaggatcttctgagcagaagcccaggcgggcccggggccttggctggcaaataaagcgttagcccgcagcgaaaaaaaaaaaaaaaaaaaaa

SEQ ID NO: 3 - DNA, 618 bp, Artificial Sequence
  Homo sapiens prolactin-induced protein(PIP)
ggggaccacttctctgggacacattgccttctgttttctccagcatgcgcttgctccagctcctgttcagggccagccctgccaccctgctcctggttctctgcctgcagttgggggccaacaaagctcaggacaacactcggaagatcataataaagaattttgacattcccaagtcagtacgtccaaatgacgaagtcactgcagtgcttgcagttcaaacagaattgaaagaatgcatggtggttaaaacttacctcattagcagcatccctctacaaggtgcatttaactataagtatactgcctgcctatgtgacgacaatccaaaaaccttctactgggacttttacaccaacagaactgtgcaaattgcagccgtcgttgatgttattcgggaattaggcatctgccctgatgatgctgctgtaatccccatcaaaaacaaccggttttatactattgaaatcctaaaggtagaataatggaagccctgtctgtttgccacacccaggtgatttcctctaaagaaacttggctggaatttctgctgtggtctataaaataaacttcttaacatgcttctacaaaaaaaaaaaaaaaaaaaaaaaaaaaaaa

SEQ ID NO: 4 - DNA, 2802 bp, Artificial Sequence
  Homo sapiens heat shock protein family A
ccagcagcaggaggcgcgcgaggcaccacggcctggcggccgagagtcagggaggaacctcatttacataacggccgcccctctgtctcctggcgggggccggagtcccgcccctcgtccaacttgaaatctgttgggtcacgggccagtcactccgacctaggcaagcctgtggtggagctggaagagtttgtgagggcggtcccgggagcggattgggtctgggagttcccagaggcggctataagaaccgggaactgggcgcggggagctgagttgctggtagtgcccgtggtgcttggttcgaggtggccgttagttgactccgcggagttcatctccctggttttcccgtcctaacgtcgctcgcctttcagtcaggatgtctgcccgtggcccggctatcggcatcgacctgggcaccacctattcgtgcgtcggggtcttccaacatggcaaggtggagatcatcgccaacgaccagggcaatcgcaccacccccagctacgtggccttcacggacaccgagcgcctcatcggcgacgccgccaagaaccaggtggccatgaaccccaccaacaccatcttcgacgccaagaggctgattggacggaaattcgaggatgccacagtgcagtcggatatgaaacactggccgttccgggtggtgagcgagggaggcaagcccaaagtgcaagtagagtacaagggggagaccaagaccttcttcccagaggagatatcctccatggtcctcacgaagatgaaggagatcgcggaagcctacctggggggcaaggtgcacagcgcggtcataacggtcccggcctatttcaacgactcgcagcgccaggccaccaaggacgcaggcaccatcacggggctcaatgtgctgcgcatcatcaacgagcccacggcggcggccatcgcctacggcctggacaagaagggctgcgcgggcggcgagaagaacgtgctcatctttgacctgggcggtggcactttcgacgtgtccatcctgaccatcgaggatggcatcttcgaggtgaagtccacggccggcgacacccacctgggcggtgaggacttcgacaaccgcatggtgagccacctggcggaggagttcaagcgcaagcacaagaaggacattgggcccaacaagcgcgccgtgaggcggctgcgcaccgcttgcgagcgcgccaagcgcaccctgagctcgtccacgcaggcgagcatcgagatcgactcgctctacgagggcgtggacttctatacgtccatcacgcgcgcccgcttcgaggagctcaatgccgacctctttcgcgggaccctggagccggtggagaaggcgctgcgcgacgccaagctggacaagggccagatccaggagatcgtgctggtgggcggctccactcgtatccccaagatccagaagctgctgcaggatttcttcaacggcaaggagctgaacaagagcatcaaccccgacgaggcggtggcctatggcgccgcggtgcaggcggccatcctcatcggcgacaaatcagagaatgtgcaggacctgctgctactcgacgtgaccccgttgtcgctgggcatcgagacagctggcggtgtcatgaccccactcatcaagaggaacaccacgatccccaccaagcagacgcagaccttcaccacctactcggacaaccagagcagcgtactggtgcaggtatacgagggcgaacgggccatgaccaaggacaataacctgctgggcaagttcgacctgaccgggattccccctgcgcctcgcggggtcccccaaatcgaggttaccttcgacattgacgccaatggcatccttaacgttaccgccgccgacaagagcaccggtaaggaaaacaaaatcaccatcaccaatgacaaaggtcgtctgagcaaggacgacattgaccggatggtgcaggaggcggagcggtacaaatcggaagatgaggcgaatcgcgaccgagtcgcggccaaaaacgccctggagtcctatacctacaacatcaagcagacggtggaagacgagaaactgaggggcaagattagcgagcaggacaaaaacaagatcctcgacaagtgtcaggaggtgatcaactggctcgaccgaaaccagatggcagagaaagatgagtatgaacacaagcagaaagagctcgaaagagtttgcaaccccatcatcagcaaactttaccaaggtggtcctggcggcggcagcggcggcggcggttcaggagcctccgggggacccaccatcgaagaagtggactaagcttgcactcaagtcagcgtaaacctctttgcctttctctctctctctttttttttgtttgtttctttgaaatgtccttgtgccaagtacgagatctattgttggaagtctttggtatatgcaaatgaaaggagaggtgcaacaacttagtttaattataaaagttccaaagtttgttttttaaaaacattattcgaggtttctctttaatgcattttgcgtgtttgctgacttgagcatttttgattagttcgtgcatggagatttgtttgagatgagaaaccttaagtttgcacacctgttctgtagaagcttggaaacagtaaaatatataggagcttaaattgtttatttttatgtactactttaaaactaaactgaacattgcagtaatgttaaggacaggtatactttttgcaaacaaatgcataaatgcaaatgtaaagtaaagctgaaattgatctcaaaaaaaaaaaaaaaaaaaaaaaaaaaaaaaaaaa

SEQ ID NO: 5 - DNA, 1017 bp, Artificial Sequence
  galectin 3 (LGALS3)
gagtatttgaggctcggagccaccgccccgccggcgcccgcagcacctcctcgccagcagccgtccggagccagccaacgagcggaaaatggcagacaatttttcgctccatgatgcgttatctgggtctggaaacccaaaccctcaaggatggcctggcgcatgggggaaccagcctgctggggcagggggctacccaggggcttcctatcctggggcctaccccgggcaggcacccccaggggcttatcctggacaggcacctccaggcgcctaccctggagcacctggagcttatcccggagcacctgcacctggagtctacccagggccacccagcggccctggggcctacccatcttctggacagccaagtgccaccggagcctaccctgccactggcccctatggcgcccctgctgggccactgattgtgccttataacctgcctttgcctgggggagtggtgcctcgcatgctgataacaattctgggcacggtgaagcccaatgcaaacagaattgctttagatttccaaagagggaatgatgttgccttccactttaacccacgcttcaatgagaacaacaggagagtcattgtttgcaatacaaagctggataataactggggaagggaagaaagacagtcggttttcccatttgaaagtgggaaaccattcaaaatacaagtactggttgaacctgaccacttcaaggttgcagtgaatgatgctcacttgttgcagtacaatcatcgggttaaaaaactcaatgaaatcagcaaactgggaatttctggtgacatagacctcaccagtgcttcatataccatgatataatctgaaaggggcagattaaaaaaaaaaaaagaatctaaaccttacatgtgtaaaggtttcatgttcactgtgagtgaaaatttttacattcatcaatatccctcttgtaagtcatctacttaataaatattacagtgaattacctgtctcaatatgtcaaaaaaaaaaaaaaaaaa

SEQ ID NO: 6 - DNA, 450 bp, Artificial Sequence
  S100 calcium binding protein A
gtccaaacacacacatctcactcatccttctactcgtgacgcttcccagctctggctttttgaaagcaaagatgagcaacactcaagctgagaggtccataataggcatgatcgacatgtttcacaaatacaccagacgtgatgacaagattgagaagccaagcctgctgacgatgatgaaggagaacttccccaacttccttagtgcctgtgacaaaaagggcacaaattacctcgccgatgtctttgagaaaaaggacaagaatgaggataagaagattgatttttctgagtttctgtccttgctgggagacatagccacagactaccacaagcagagccatggagcagcgccctgttccgggggcagccagtgacccagccccaccaatgggcctccagagaccccaggaacaataaaatgtcttctcccaccagaaaaaaaaaaaa

SEQ ID NO: 7 - DNA, 1254 bp, Artificial Sequence
  Lysosome-associated membrane glycoprotein 1
atggcggcccccggcagcgcccggcgacccctgctgctgctactgctgttgctgctgctcggcctcatgcattgtgcgtcagcagcaatgtttatggtgaaaaatggcaacgggaccgcgtgcataatggccaacttctctgctgccttctcagtgaactacgacaccaagagtggccctaagaacatgacctttgacctgccatcagatgccacagtggtgctcaaccgcagctcctgtggaaaagagaacacttctgaccccagtctcgtgattgcttttggaagaggacatacactcactctcaatttcacgagaaatgcaacacgttacagcgtccagctcatgagttttgtttataacttgtcagacacacaccttttccccaatgcgagctccaaagaaatcaagactgtggaatctataactgacatcagggcagatatagataaaaaatacagatgtgttagtggcacccaggtccacatgaacaacgtgaccgtaacgctccatgatgccaccatccaggcgtacctttccaacagcagcttcagccggggagagacacgctgtgaacaagacaggccttccccaaccacagcgccccctgcgccacccagcccctcgccctcacccgtgcccaagagcccctctgtggacaagtacaacgtgagcggcaccaacgggacctgcctgctggccagcatggggctgcagctgaacctcacctatgagaggaaggacaacacgacggtgacaaggcttctcaacatcaaccccaacaagacctcggccagcgggagctgcggcgcccacctggtgactctggagctgcacagcgagggcaccaccgtcctgctcttccagttcgggatgaatgcaagttctagccggtttttcctacaaggaatccagttgaatacaattcttcctgacgccagagaccctgcctttaaagctgccaacggctccctgcgagcgctgcaggccacagtcggcaattcctacaagtgcaacgcggaggagcacgtccgtgtcacgaaggcgttttcagtcaatatattcaaagtgtgggtccaggctttcaaggtggaaggtggccagtttggctctgtggaggagtgtctgctggacgagaacagcatgctgatccccatcgctgtgggtggtgccctggcggggctggtcctcatcgtcctcatcgcctacctcgtcggcaggaagaggagtcacgcaggctaccagactatctag

SEQ ID NO: 8 - DNA, 1278 bp, Artificial Sequence
  Serpin B12
atggactctcttgttacagcaaacaccaaattttgctttgatctttttcaagagataggcaaagatgatcgtcataaaaacatatttttctctcccctgagcctctcagctgcccttggtatggtacgcttgggtgctagaagtgacagtgcacatcagattgatgaggtactacacttcaacgaattttcccagaatgaaagcaaagaacctgacccttgtctgaaaagcaacaaacaaaaagtgctggctgacagctctctggaggggcagaaaaaaacgacagagcctctggatcagcaggctgggtccttaaacaatgagagcggactggtcagctgctactttgggcagcttctctccaaattagacaggatcaagactgattacacactgagtattgccaacaggctttatggagagcaggaattcccaatctgtcaggaatacttagatggtgtgattcaattttaccacacgacgattgaaagtgttgatttccaaaaaaaccctgaaaaatccagacaagagattaacttctgggttgaatgtcaatcccaaggtaaaatcaaggaactcttcagcaaggacgctattaatgctgagactgtgctggtactggtgaatgctgtttacttcaaggccaaatgggaaacatactttgaccatgaaaacacggtggatgcacctttctgtctaaatgcgaatgaaaacaagagtgtgaagatgatgacgcaaaaaggcctctacagaattggcttcatagaggaggtgaaggcacagatcctggaaatgaggtacaccaaggggaagctcagcatgttcgtgctgctgccatctcactctaaagataacctgaagggtctggaagagcttgaaaggaaaatcacctatgaaaaaatggtggcctggagcagctcagaaaacatgtcagaagaatcggtggtcctgtccttcccccggttcaccctggaagacagctatgatctcaattccattttacaagacatgggcattacggatatctttgatgaaacgagggctgatcttactggaatctctccaagtcccaatttgtacttgtcaaaaattatccacaaaacctttgtggaggtggatgaaaacggtacccaggcagctgcagccactggggctgttgtctcggaaaggtcactacgatcttgggtggagtttaatgccaaccacccttttctctttttcattagacacaacaaaacccaaaccattctcttttatggcagggtctgctctccttaa

SEQ ID NO: 9 - DNA, 2132 bp, Artificial Sequence
  Lactotransferrin
tgaaacttgtcttcctcgtcctgctgttcctcggggccctcggactgtgtctggctggccgtaggaggagtgttcagtggtgcgccgtatcccaacccgaggccacaaaatgcttccaatggcaaaggaatatgagaaaagtgcgtggccctcctgtcagctgcataaagagagactcccccatccagtgtatccaggccattgcggaaaacagggccgatgctgtgacccttgatggtggtttcatatacgaggcaggcctggccccctacaaactgcgacctgtagcggcggaagtctacgggaccgaaagacagccacgaactcactattatgccgtggctgtggtgaagaagggcggcagctttcagctgaacgaactgcaaggtctgaagtcctgccacacaggccttcgcaggaccgctggatggaatgtccctatagggacacttcgtccattcttgaattggacgggtccacctgagcccattgaggcagctgtggccaggttcttctcagccagctgtgttcccggtgcagataaaggacagttccccaacctgtgtcgcctgtgtgcggggacaggggaaaacaaatgtgccttctcctcccaggaaccgtacttcagctactctggtgccttcaagtgtctgagagacggggctggagacgtggcttttatcagagagagcacagtgtttgaggacctgtcagacgaggctgaaagggacgagtatgagttactctgcccagacaacactcggaagccagtggacaagttcaaagactgccatctggcccgggtcccttctcatgccgttgtggcacgaagtgtgaatggcaaggaggatgccatctggaatcttctccgccaggcacaggaaaagtttggaaaggacaagtcaccgaaattccagctctttggctcccctagtgggcagaaagatctgctgttcaaggactctgccattgggttttcgagggtgcccccgaggatagattctgggctgtaccttggctccggctacttcactgccatccagaacttgaggaaaagtgaggaggaagtggctgcccggcgtgcgcgggtcgtgtggtgtgcggtgggcgagcaggagctgcgcaagtgtaaccagtggagtggcttgagcgaaggcagcgtgacctgctcctcggcctccaccacagaggactgcatcgccctggtgctgaaaggagaagctgatgccatgagtttggatggaggatatgtgtacactgcaggcaaatgtggtttggtgcctgtcctggcagagaactacaaatcccaacaaagcagtgaccctgatcctaactgtgtggatagacctgtggaaggatatcttgctgtggcggtggttaggagatcagacactagccttacctggaactctgtgaaaggcaagaagtcctgccacaccgccgtggacaggactgcaggctggaatatccccatgggcctgctcttcaaccagacgggctcctgcaaatttgatgaatatttcagtcaaagctgtgcccctgggtctgacccgagatctaatctctgtgctctgtgtattggcgacgagcagggtgagaataagtgcgtgcccaacagcaacgagagatactacggctacactggggctttccggtgcctggctgagaatgctggagacgttgcatttgtgaaagatgtcactgtcttgcagaacactgatggaaataacaatgaggcatgggctaaggatttgaagctggcagactttgcgctgctgtgcctcgatggcaaacggaagcctgtgactgaggctagaagctgccatcttgccatggccccgaatcatgccgtggtgtctcggatggataaggtggaacgcctgaaacaggtgttgctccaccaacaggctaaatttgggagaaatggatctgactgcccggacaagttttgcttattccagtctgaaaccaaaaaccttctgttcaatgacaacactgagtgtctggccagactccatggcaaaacaacatatgaaaaatatttgggaccacagtatgtcgcaggcattactaatctgaaaaagtgctcaacctcccccctcctggaagcctgtgaattcctcaggaagtaa

SEQ ID NO: 10 - DNA, 606 bp, Artificial Sequence
  Alpha-1-acid glycoprotein 1
atggcgctgtcctgggttcttacagtcctgagcctcctacctctgctggaagcccagatcccattgtgtgccaacctagtaccggtgcccatcaccaacgccaccctggaccggatcactggcaagtggttttatatcgcatcggcctttcgaaacgaggagtacaataagtcggttcaggagatccaagcaaccttcttttacttcacccccaacaagacagaggacacgatctttctcagagagtaccagacccgacaggaccagtgcatctataacaccacctacctgaatgtccagcgggaaaatgggaccatctccagatacgtgggaggccaagagcatttcgctcacttgctgatcctcagggacaccaagacctacatgcttgcttttgacgtgaacgatgagaagaactgggggctgtctgtctatgctgacaagccagagacgaccaaggagcaactgggagagttctacgaagctctcgactgcttgcgcattcccaagtcagatgtcgtgtacaccgattggaaaaaggataagtgtgagccactggagaagcagcacgagaaggagaggaaacaggaggagggggaatcctag

SEQ ID NO: 11 - DNA, 1044 bp, Artificial Sequence
  CD5 antigen-like
atggctctgctattctccttgatccttgccatttgcaccagacctggattcctagcgtctccatctggagtgcggctggtggggggcctccaccgctgtgaagggcgggtggaggtggaacagaaaggccagtggggcaccgtgtgtgatgacggctgggacattaaggacgtggctgtgttgtgccgggagctgggctgtggagctgccagcggaacccctagtggtattttgtatgagccaccagcagaaaaagagcaaaaggtcctcatccaatcagtcagttgcacaggaacagaagatacattggctcagtgtgagcaagaagaagtttatgattgttcacatgatgaagatgctggggcatcgtgtgagaacccagagagctctttctccccagtcccagagggtgtcaggctggctgacggccctgggcattgcaagggacgcgtggaagtgaagcaccagaaccagtggtataccgtgtgccagacaggctggagcctccgggccgcaaaggtggtgtgccggcagctgggatgtgggagggctgtactgactcaaaaacgctgcaacaagcatgcctatggccgaaaacccatctggctgagccagatgtcatgctcaggacgagaagcaacccttcaggattgcccttctgggccttgggggaagaacacctgcaaccatgatgaagacacgtgggtcgaatgtgaagatccctttgacttgagactagtaggaggagacaacctctgctctgggcgactggaggtgctgcacaagggcgtatggggctctgtctgtgatgacaactggggagaaaaggaggaccaggtggtatgcaagcaactgggctgtgggaagtccctctctccctccttcagagaccggaaatgctatggccctggggttggccgcatctggctggataatgttcgttgctcaggggaggagcagtccctggagcagtgccagcacagattttgggggtttcacgactgcacccaccaggaagatgtggctgtcatctgctcaggatag

SEQ ID NO: 12 - DNA, 5235 bp, Artificial Sequence
  Complement C4-B
atgaggctgctctgggggctgatctgggcatccagcttcttcaccttatctctgcagaagcccaggttgctcttgttctctccttctgtggttcatctgggggtccccctatcggtgggggtgcagctccaggatgtgccccgaggacaggtagtgaaaggatcagtgttcctgagaaacccatctcgtaataatgtcccctgctccccaaaggtggacttcacccttagctcagaaagagacttcgcactcctcagtctccaggtgcccttgaaagatgcgaagagctgtggcctccatcaactcctcagaggccctgaggtccagctggtggcccattcgccatggctaaaggactctctgtccagaacgacaaacatccagggtatcaacctgctcttctcctctcgccgggggcacctctttttgcagacggaccagcccatttacaaccctggccagcgggttcggtaccgggtctttgctctggatcagaagatgcgcccgagcactgacaccatcacagtcatggtggagaactctcacggcctccgcgtgcggaagaaggaggtgtacatgccctcgtccatcttccaggatgactttgtgatcccagacatctcagagccagggacctggaagatctcagcccgattctcagatggcctggaatccaacagcagcacccagtttgaggtgaagaaatatgtccttcccaactttgaggtgaagatcacccctggaaagccctacatcctgacggtgccaggccatcttgatgaaatgcagttagacatccaggccaggtacatctatgggaagccagtgcagggggtggcatatgtgcgctttgggctcctagatgaggatggtaagaagactttctttcgggggctggagagtcagaccaagctggtgaatggacagagccacatttccctctcaaaggcagagttccaggacgccctggagaagctgaatatgggcattactgacctccaggggctgcgcctctacgttgctgcagccatcattgagtctccaggtggggagatggaggaggcagagctcacatcctggtattttgtgtcatctcccttctccttggatcttagcaagaccaagcgacaccttgtgcctggggcccccttcctgctgcaggccttggtccgtgagatgtcaggctccccagcttctggcattcctgtcaaagtttctgccacggtgtcttctcctgggtctgttcctgaagtccaggacattcagcaaaacacagacgggagcggccaagtcagcattccaataattatccctcagaccatctcagagctgcagctctcagtatctgcaggctccccacatccagcgatagccaggctcactgtggcagccccaccttcaggaggccccgggtttctgtctattgagcggccggattctcgacctcctcgtgttggggacactctgaacctgaacttgcgagccgtgggcagtggggccaccttttctcattactactacatgatcctatcccgagggcagatcgtgttcatgaatcgagagcccaagaggaccctgacctcggtctcggtgtttgtggaccatcacctggcaccctccttctactttgtggccttctactaccatggagaccacccagtggccaactccctgcgagtggatgtccaggctggggcctgcgagggcaagctggagctcagcgtggacggtgccaagcagtaccggaacggggagtccgtgaagctccacttagaaaccgactccctagccctggtggcgctgggagccttggacacagctctgtatgctgcaggcagcaagtcccacaagcccctcaacatgggcaaggtctttgaagctatgaacagctatgacctcggctgtggtcctgggggtggggacagtgcccttcaggtgttccaggcagcgggcctggccttttctgatggagaccagtggaccttatccagaaagagactaagctgtcccaaggagaagacaacccggaaaaagagaaacgtgaacttccaaaaggcgattaatgagaaattgggtcagtatgcttccccgacagccaagcgctgctgccaggatggggtgacacgtctgcccatgatgcgttcctgcgagcagcgggcagcccgcgtgcagcagccggactgccgggagcccttcctgtcctgctgccaatttgctgagagtctgcgcaagaagagcagggacaagggccaggcgggcctccaacgagccctggagatcctgcaggaggaggacctgattgatgaggatgacattcccgtgcgcagcttcttcccagagaactggctctggagagtggaaacagtggaccgctttcaaatattgacactgtggctccccgactctctgaccacgtgggagatccatggcctgagcctgtccaaaaccaaaggcctatgtgtggccaccccagtccagctccgggtgttccgcgagttccacctgcacctccgcctgcccatgtctgtccgccgctttgagcagctggagctgcggcctgtcctctataactacctggataaaaacctgactgtgagcgtccacgtgtccccagtggaggggctgtgcctggctgggggcggagggctggcccagcaggtgctggtgcctgcgggctctgcccggcctgttgccttctctgtggtgcccacggcagccaccgctgtgtctctgaaggtggtggctcgagggtccttcgaattccctgtgggagatgcggtgtccaaggttctgcagattgagaaggaaggggccatccatagagaggagctggtctatgaactcaaccccttggaccaccgaggccggaccttggaaatacctggcaactctgatcccaatatgatccctgatggggactttaacagctacgtcagggttacagcctcagatccattggacactttaggctctgagggggccttgtcaccaggaggcgtggcctccctcttgaggcttcctcgaggctgtggggagcaaaccatgatctacttggctccgacactggctgcttcccgctacctggacaagacagagcagtggagcacactgcctcccgagaccaaggaccacgccgtggatctgatccagaaaggctacatgcggatccagcagtttcggaaggcggatggttcctatgcggcttggttgtcacggggcagcagcacctggctcacagcctttgtgttgaaggtcctgagtttggcccaggagcaggtaggaggctcgcctgagaaactgcaggagacatctaactggcttctgtcccagcagcaggctgacggctcgttccaggacctctctccagtgatacataggagcatgcaggggggtttggtgggcaatgatgagactgtggcactcacagcctttgtgaccatcgcccttcatcatgggctggccgtcttccaggatgagggtgcagagccattgaagcagagagtggaagcctccatctcaaaggcaagctcatttttgggggagaaagcaagtgctgggctcctgggtgcccacgcagctgccatcacggcctatgccctgacactgaccaaggcccctgcggacctgcggggtgttgcccacaacaacctcatggcaatggcccaggagactggagataacctgtactggggctcagtcactggttctcagagcaatgccgtgtcgcccaccccggctcctcgcaacccatccgaccccatgccccaggccccagccctgtggattgaaaccacagcctacgccctgctgcacctcctgcttcacgagggcaaagcagagatggcagaccaggctgcggcctggctcacccgtcagggcagcttccaagggggattccgcagtacccaagacacggtgattgccctggatgccctgtctgcctactggattgcctcccacaccactgaggagaggggtctcaatgtgactctcagctccacaggccggaatgggttcaagtcccacgcgctgcagctgaacaaccgccagattcgcggcctggaggaggagctgcagttttccttgggcagcaagatcaatgtgaaggtgggaggaaacagcaaaggaaccctgaaggtccttcgtacctacaatgtcctggacatgaagaacacgacctgccaggacctacagatagaagtgacagtcaaaggccacgtcgagtacacgatggaagcaaacgaggactatgaggactatgagtacgatgagcttccagccaaggatgacccagatgcccctctgcagcccgtgacacccctgcagctgtttgagggtcggaggaaccgccgcaggagggaggcgcccaaggtggtggaggagcaggagtccagggtgcactacaccgtgtgcatctggcggaacggcaaggtggggctgtctggcatggccatcgcggacgtcaccctcctgagtggattccacgccctgcgtgctgacctggagaagctgacctccctctctgaccgttacgtgagtcactttgagaccgaggggccccacgtcctgctgtattttgactcggtccccacctcccgggagtgcgtgggctttgaggctgtgcaggaagtgccggtggggctggtgcagccggccagcgcaaccctgtacgactactacaaccccgagcgcagatgttctgtgttttacggggcaccaagtaagagcagactcttggccaccttgtgttctgctgaagtctgccagtgtgctgaggggaagtgccctcgccagcgtcgcgccctggagcggggtctgcaggacgaggatggctacaggatgaagtttgcctgctactacccccgtgtggagtacggcttccaggttaaggttctccgagaagacagcagagctgctttccgcctctttgagaccaagatcacccaagtcctgcacttcaccaaggatgtcaaggccgctgctaatcagatgcgcaacttcctggttcgagcctcctgccgccttcgcttggaacctgggaaagaatatttgatcatgggtctggatggggccacctatgacctcgagggacacccccagtacctgctggactcgaatagctggatcgaggagatgccctctgaacgcctgtgccggagcacccgccagcgggcagcctgtgcccagctcaacgacttcctccaggagtatggcactcaggggtgccaggtgtga

SEQ ID NO: 13 - DNA, 2208 bp, Artificial Sequence
  Mannan-binding lectin serine protease 1
atgagacctacattcatgtctttcaggtggctgcttctctattatgctctgtgcttctccctgtcaaaggcttcagcccacaccgtggagctaaacaatatgtttggccagatccagtcgcctggttatccagactcctatcccagtgattcagaggtgacttggaatatcactgtcccagatgggtttcggatcaagctttacttcatgcacttcaacttggaatcctcctacctttgtgaatatgactatgtgaaggtagaaactgaggaccaggtgctggcaaccttctgtggcagggagaccacagacacagagcagactcccggccaggaggtggtcctctcccctggctccttcatgtccatcactttccggtcagatttctccaatgaggagcgtttcacaggctttgatgcccactacatggctgtggatgtggacgagtgcaaggagagggaggacgaggagctgtcctgtgaccactactgccacaactacattggcggctactactgctcctgccgcttcggctacatcctccacacagacaacaggacctgccgagtggagtgcagtgacaacctcttcactcaaaggactggggtgatcaccagccctgacttcccaaacccttaccccaagagctctgaatgcctgtataccatcgagctggaggagggtttcatggtcaacctgcagtttgaggacatatttgacattgaggaccatcctgaggtgccctgcccctatgactacatcaagatcaaagttggtccaaaagttttggggcctttctgtggagagaaagccccagaacccatcagcacccagagccacagtgtcctgatcctgttccatagtgacaactcgggagagaaccggggctggaggctctcatacagggctgcaggaaatgagtgcccagagctacagcctcctgtccatgggaaaatcgagccctcccaagccaagtatttcttcaaagaccaagtgctcgtcagctgtgacacaggctacaaagtgctgaaggataatgtggagatggacacattccagattgagtgtctgaaggatgggacgtggagtaacaagattcccacctgtaaaattgtagactgtagagccccaggagagctggaacacgggctgatcaccttctctacaaggaacaacctcaccacatacaagtctgagatcaaatactcctgtcaggagccctattacaagatgctcaacaataacacaggtatatatacctgttctgcccaaggagtctggatgaataaagtattggggagaagcctacccacctgccttccagagtgtggtcagccctcccgctccctgccaagcctggtcaagaggatcattgggggccgaaatgctgagcctggcctcttcccgtggcaggccctgatagtggtggaggacacttcgagagtgccaaatgacaagtggtttgggagtggggccctgctctctgcgtcctggatcctcacagcagctcatgtgctgcgctcccagcgtagagacaccacggtgataccagtctccaaggagcatgtcaccgtctacctgggcttgcatgatgtgcgagacaaatcgggggcagtcaacagctcagctgcccgagtggtgctccacccagacttcaacatccaaaactacaaccacgatatagctctggtgcagctgcaggagcctgtgcccctgggaccccacgttatgcctgtctgcctgccaaggcttgagcctgaaggcccggccccccacatgctgggcctggtggccggctggggcatctccaatcccaatgtgacagtggatgagatcatcagcagtggcacacggaccttgtcagatgtcctgcagtatgtcaagttacccgtggtgcctcacgctgagtgcaaaactagctatgagtcccgctcgggcaattacagcgtcacggagaacatgttctgtgctggctactacgagggcggcaaagacacgtgccttggagatagcggtggggcctttgtcatctttgatgacttgagccagcgctgggtggtgcaaggcctggtgtcctgggggggacctgaagaatgcggcagcaagcaggtctatggagtctacacaaaggtctccaattacgtggactgggtgtgggagcagatgggcttaccacaaagtgttgtggagccccaggtggaacggtga

SEQ ID NO: 14 - DNA, 741 bp, Artificial Sequence
  Proteasome subunit alpha type-6
atgtcccgtggttccagcgccggttttgaccgccacattaccattttttcacccgagggtcggctctaccaagtagaatatgcttttaaggctattaaccagggtggccttacatcagtagctgtcagagggaaagactgtgcagtaattgtcacacagaagaaagtacctgacaaattattggattccagcacagtgactcacttattcaagataactgaaaacattggttgtgtgatgaccggaatgacagctgacagcagatcccaggtacagagggcacgctatgaggcagctaactggaaatacaagtatggctatgagattcctgtggacatgctgtgtaaaagaattgccgatatttctcaggtctacacacagaatgctgaaatgaggcctcttggttgttgtatgattttaattggtatagatgaagagcaaggccctcaggtatataagtgtgatcctgcaggttactactgtgggtttaaagccactgcagcgggagttaaacaaactgagtcaaccagcttccttgaaaaaaaagtgaagaagaaatttgattggacatttgaacagacagtggaaactgcaattacatgcctgtctactgttctatcaattgatttcaaaccttcagaaatagaagttggagtagtgacagttgaaaatcctaaattcaggattcttacagaagcagagattgatgctcaccttgttgctctagcagagagagactaa

SEQ ID NO: 15 - DNA, 600 bp, Artificial Sequence
  Peroxiredoxin-1
atgtcttcaggaaatgctaaaattgggcaccctgcccccaacttcaaagccacagctgttatgccagatggtcagtttaaagatatcagcctgtctgactacaaaggaaaatatgttgtgttcttcttttaccctcttgacttcacctttgtgtgccccacggagatcattgctttcagtgatagggcagaagaatttaagaaactcaactgccaagtgattggtgcttctgtggattctcacttctgtcatctagcatgggtcaatacacctaagaaacaaggaggactgggacccatgaacattcctttggtatcagacccgaagcgcaccattgctcaggattatggggtcttaaaggctgatgaaggcatctcgttcaggggcctttttatcattgatgataagggtattcttcggcagatcactgtaaatgacctccctgttggccgctctgtggatgagactttgagactagttcaggccttccagttcactgacaaacatggggaagtgtgcccagctggctggaaacctggcagtgataccatcaagcctgatgtccaaaagagcaaagaatatttctccaagcagaagtga

SEQ ID NO: 16 - DNA, 285 bp, Artificial Sequence
  Neutrophil defensin 3
atgaggaccctcgccatccttgctgccattctcctggtggccctgcaggcccaggctgagccactccaggcaagagctgatgaggttgctgcagccccggagcagattgcagcggacatcccagaagtggttgtttcccttgcatgggacgaaagcttggctccaaagcatccaggctcaaggaaaaacatggactgctattgcagaataccagcgtgcattgcaggagaacgtcgctatggaacctgcatctaccagggaagactctgggcattctgctgctga

SEQ ID NO: 17 - DNA, 2232 bp, Artificial Sequence
  CD44 antigen
atggacaagttttggtggcacgcagcctggggactctgcctcgtgccgctgagcctggcgcagatcgatttgaatataacctgccgctttgcaggtgtattccacgtggagaaaaatggtcgctacagcatctctcggacggaggccgctgacctctgcaaggctttcaatagcaccttgcccacaatggcccagatggagaaagctctgagcatcggatttgagacctgcaggtatgggttcatagaagggcacgtggtgattccccggatccaccccaactccatctgtgcagcaaacaacacaggggtgtacatcctcacatccaacacctcccagtatgacacatattgcttcaatgcttcagctccacctgaagaagattgtacatcagtcacagacctgcccaatgcctttgatggaccaattaccataactattgttaaccgtgatggcacccgctatgtccagaaaggagaatacagaacgaatcctgaagacatctaccccagcaaccctactgatgatgacgtgagcagcggctcctccagtgaaaggagcagcacttcaggaggttacatcttttacaccttttctactgtacaccccatcccagacgaagacagtccctggatcaccgacagcacagacagaatccctgctaccactttgatgagcactagtgctacagcaactgagacagcaaccaagaggcaagaaacctgggattggttttcatggttgtttctaccatcagagtcaaagaatcatcttcacacaacaacacaaatggctggtacgtcttcaaataccatctcagcaggctgggagccaaatgaagaaaatgaagatgaaagagacagacacctcagtttttctggatcaggcattgatgatgatgaagattttatctccagcaccatttcaaccacaccacgggcttttgaccacacaaaacagaaccaggactggacccagtggaacccaagccattcaaatccggaagtgctacttcagacaaccacaaggatgactgcagatgtagacagaaatggcaccactgcttatgaaggaaactggaacccagaagcacaccctcccctcattcaccatgagcatcatgaggaagaagagaccccacattctacaagcacaatccaggcaactcctagtagtacaacggaagaaacagctacccagaaggaacagtggtttggcaacagatggcatgagggatatcgccaaacacccaaagaagactcccattcgacaacagggacagctgcagcctcagctcataccagccatccaatgcaaggaaggacaacaccaagcccagaggacagttcctggactgatttcttcaacccaatctcacaccccatgggacgaggtcatcaagcaggaagaaggatggatatggactccagtcatagtataacgcttcagcctactgcaaatccaaacacaggtttggtggaagatttggacaggacaggacctctttcaatgacaacgcagcagagtaattctcagagcttctctacatcacatgaaggcttggaagaagataaagaccatccaacaacttctactctgacatcaagcaataggaatgatgtcacaggtggaagaagagacccaaatcattctgaaggctcaactactttactggaaggttatacctctcattacccacacacgaaggaaagcaggaccttcatcccagtgacctcagctaagactgggtcctttggagttactgcagttactgttggagattccaactctaatgtcaatcgttccttatcaggagaccaagacacattccaccccagtggggggtcccataccactcatggatctgaatcagatggacactcacatgggagtcaagaaggtggagcaaacacaacctctggtcctataaggacaccccaaattccagaatggctgatcatcttggcatccctcttggccttggctttgattcttgcagtttgcattgcagtcaacagtcgaagaaggtgtgggcagaagaaaaagctagtgatcaacagtggcaatggagctgtggaggacagaaagccaagtggactcaacggagaggccagcaagtctcaggaaatggtgcatttggtgaacaaggagtcgtcagaaactccagaccagtttatgacagctgatgagacaaggaacctgcagaatgtggacatgaagattggggtgtaa

SEQ ID NO: 18 - DNA, 993 bp, Artificial Sequence
  Arginase-1
atgagcgccaagtccagaaccatagggattattggagctcctttctcaaagggacagccacgaggaggggtggaagaaggccctacagtattgagaaaggctggtctgcttgagaaacttaaagaacaagtaactcaaaactttttaattttagagtgtgatgtgaaggattatggggacctgccctttgctgacatccctaatgacagtccctttcaaattgtgaagaatccaaggtctgtgggaaaagcaagcgagcagctggctggcaaggtggcagaagtcaagaagaacggaagaatcagcctggtgctgggcggagaccacagtttggcaattggaagcatctctggccatgccagggtccaccctgatcttggagtcatctgggtggatgctcacactgatatcaacactccactgacaaccacaagtggaaacttgcatggacaacctgtatctttcctcctgaaggaactaaaaggaaagattcccgatgtgccaggattctcctgggtgactccctgtatatctgccaaggatattgtgtatattggcttgagagacgtggaccctggggaacactacattttgaaaactctaggcattaaatacttttcaatgactgaagtggacagactaggaattggcaaggtgatggaagaaacactcagctatctactaggaagaaagaaaaggccaattcatctaagttttgatgttgacggactggacccatctttcacaccagctactggcacaccagtcgtgggaggtctgacatacagagaaggtctctacatcacagaagaaatctacaaaacagggctactctcaggattagatataatggaagtgaacccatccctggggaagacaccagaagaagtaactcgaacagtgaacacagcagttgcaataaccttggcttgtttcggacttgctcgggagggtaatcacaagcctattgactaccttaacccacctaagtaa